European Patent Specification EP 3 505 620 B1, published July 26, 2023. Title: METHOD FOR PRODUCING HUMAN DIARRHEA VIRUS. Applicant: KEIO UNIVERSITY. The sequence listing filed with the application follows.

SEQUENCE LISTING (3 sequences)

SEQ ID NO: 1 - DNA, 26 bp, Artificial Sequence
  sense primer named COG2F
  misc_feature (9)..(9): n is a, c, g, or t
cargarbcnatgttyagrtggatgag

SEQ ID NO: 2 - DNA, 21 bp, Artificial Sequence
  antisense primer named COG2R
tcgacgccatcttcattcaca

SEQ ID NO: 3 - DNA, 20 bp, Artificial Sequence
  synthesyzed probe for RING2
tgggagggcgatcgcaatct